European Patent Specification EP 3 060 669 B1, published December 11, 2024. Title: Treatment of neurological diseases using adeno-associated virus (AAV) comprising   AAV-5 capsid proteins. Applicant: uniQure IP B.V. The sequence listing filed with the application follows.

SEQUENCE LISTING (7 sequences)

SEQ ID NO: 1 - DNA, 145 bp, adeno-associated virus 2
ttggccactccctctctgcgcgctcgctcgctcactgaggccgggcgaccaaaggtcgcccgacgcccgggctttgcccgggcggcctcagtgagcgagcgagcgcgcagagagggagtggccaactccatcactaggggttcct

SEQ ID NO: 2 - DNA, 183 bp, adeno-associated virus 2
gcgcggtaccccatggaggaacccctagtgatggagttggccactccctctctgcgcgctcgctcgctcactgaggccgcccgggcaaagcccgggcgtcgggcgacctttggtcgcccggcctcagtgagcgagcgagcgcgcagagagggagtggccaagatatcccatggggtaccgcgc

SEQ ID NO: 3 - DNA, 2203 bp, adeno-associated virus 5
atgtcttttgttgatcaccctccagattggttggaagaagttggtgaaggtcttcgcgagtttttgggccttgaagcgggcccaccgaaaccaaaacccaatcagcagcatcaagatcaagcccgtggtcttgtgctgcctggttataactatctcggacccggaaacggtctcgatcgaggagagcctgtcaacagggcagacgaggtcgcgcgagagcacgacatctcgtacaacgagcagcttgaggcgggagacaacccctacctcaagtacaaccacgcggacgccgagtttcaggagaagctcgccgacgacacatccttcgggggaaacctcggaaaggcagtctttcaggccaagaaaagggttctcgaaccttttggcctggttgaagagggtgctaagacggcccctaccggaaagcggatagacgaccactttccaaaaagaaagaaggctcggaccgaagaggactccaagccttccacctcgtcagacgccgaagctggacccagcggatcccagcagctgcaaatcccagcccaaccagcctcaagtttgggagctgatacaatgtctgcgggaggtggcggcccattgggcgacaataaccaaggtgccgatggagtgggcaatgcctcgggagattggcattgcgattccacgtggatgggggacagagtcgtcaccaagtccacccgaacctgggtgctgcccagctacaacaaccaccagtaccgagagatcaaaagcggctccgtcgacggaagcaacgccaacgcctactttggatacagcaccccctgggggtactttgactttaaccgcttccacagccactggagcccccgagactggcaaagactcatcaacaactactggggcttcagaccccggtccctcagagtcaaaatcttcaacattcaagtcaaagaggtcacggtgcaggactccaccaccaccatcgccaacaacctcacctccaccgtccaagtgtttacggacgacgactaccagctgccctacgtcgtcggcaacgggaccgagggatgcctgccggccttccctccgcaggtctttacgctgccgcagtacggttacgcgacgctgaaccgcgacaacacagaaaatcccaccgagaggagcagcttcttctgcctagagtactttcccagcaagatgctgagaacgggcaacaactttgagtttacctacaactttgaggaggtgcccttccactccagcttcgctcccagtcagaacctgttcaagctggccaacccgctggtggaccagtacttgtaccgcttcgtgagcacaaataacactggcggagtccagttcaacaagaacctggccgggagatacgccaacacctacaaaaactggttcccggggcccatgggccgaacccagggctggaacctgggctccggggtcaaccgcgccagtgtcagcgccttcgccacgaccaataggatggagctcgagggcgcgagttaccaggtgcccccgcagccgaacggcatgaccaacaacctccagggcagcaacacctatgccctggagaacactatgatcttcaacagccagccggcgaacccgggcaccaccgccacgtacctcgagggcaacatgctcatcaccagcgagagcgagacgcagccggtgaaccgcgtggcgtacaacgtcggcgggcagatggccaccaacaaccagagctccaccactgcccccgcgaccggcacgtacaacctccaggaaatcgtgcccggcagcgtgtggatggagagggacgtgtacctccaaggacccatctgggccaagatcccagagacgggggcgcactttcacccctctccggccatgggcggattcggactcaaacacccaccgcccatgatgctcatcaagaacacgcctgtgcccggaaatatcaccagcttctcggacgtgcccgtcagcagcttcatcacccagtacagcaccgggcaggtcaccgtggagatggagtgggagctcaagaaggaaaactccaagaggtggaacccagagatccagtacacaaacaactacaacgacccccagtttgtggactttgccccggacagcaccggggaatacagaaccaccagacctatcggaacccgataccttacccgacccctttaacccattcatgtcgcataccctcaataaa

SEQ ID NO: 4 - protein, 724 aa, adeno-associated virus 5
MSFVDHPPDWLEEVGEGLREFLGLEAGPPKPKPNQQHQDQARGLVLPGYNYLGPGNGLDRGEPVNRADEVAREHDISYNEQLEAGDNPYLKYNHADAEFQEKLADDTSFGGNLGKAVFQAKKRVLEPFGLVEEGAKTAPTGKRIDDHFPKRKKARTEEDSKPSTSSDAEAGPSGSQQLQIPAQPASSLGADTMSAGGGGPLGDNNQGADGVGNASGDWHCDSTWMGDRVVTKSTRTWVLPSYNNHQYREIKSGSVDGSNANAYFGYSTPWGYFDFNRFHSHWSPRDWQRLINNYWGFRPRSLRVKIFNIQVKEVTVQDSTTTIANNLTSTVQVFTDDDYQLPYVVGNGTEGCLPAFPPQVFTLPQYGYATLNRDNTENPTERSSFFCLEYFPSKMLRTGNNFEFTYNFEEVPFHSSFAPSQNLFKLANPLVDQYLYRFVSTNNTGGVQFNKNLAGRYANTYKNWFPGPMGRTQGWNLGSGVNRASVSAFATTNRMELEGASYQVPPQPNGMTNNLQGSNTYALENTMIFNSQPANPGTTATYLEGNMLITSESETQPVNRVAYNVGGQMATNNQSSTTAPATGTYNLQEIVPGSVWMERDVYLQGPIWAKIPETGAHFHPSPAMGGFGLKHPPPMMLIKNTPVPGNITSFSDVPVSSFITQYSTGQVTVEMEWELKKENSKRWNPEIQYTNNYNDPQFVDFAPDSTGEYRTTRPIGTRYLTRPL

SEQ ID NO: 5 - DNA, 1876 bp, adeno-associated virus 2
  CDS (11)..(1876)
cgcagccgccatgccggggttttacgagattgtgattaaggtccccagcgaccttgacgagcatctgcccggcatttctgacagctttgtgaactgggtggccgagaaggaatgggagttgccgccagattctgacatggatctgaatctgattgagcaggcacccctgaccgtggccgagaagctgcagcgcgactttctgacggaatggcgccgtgtgagtaaggccccggaggcccttttctttgtgcaatttgagaagggagagagctacttccacatgcacgtgctcgtggaaaccaccggggtgaaatccatggttttgggacgtttcctgagtcagattcgcgaaaaactgattcagagaatttaccgcgggatcgagccgactttgccaaactggttcgcggtcacaaagaccagaaatggcgccggaggcgggaacaaggtggtggatgagtgctacatccccaattacttgctccccaaaacccagcctgagctccagtgggcgtggactaatatggaacagtatttaagcgcctgtttgaatctcacggagcgtaaacggttggtggcgcagcatctgacgcacgtgtcgcagacgcaggagcagaacaaagagaatcagaatcccaattctgatgcgccggtgatcagatcaaaaacttcagccaggtacatggagctggtcgggtggctcgtggacaaggggattacctcggagaagcagtggatccaggaggaccaggcctcatacatctccttcaatgcggcctccaactcgcggtcccaaatcaaggctgccttggacaatgcgggaaagattatgagcctgactaaaaccgcccccgactacctggtgggccagcagcccgtggaggacatttccagcaatcggatttataaaattttggaactaaacgggtacgatccccaatatgcggcttccgtctttctgggatgggccacgaaaaagttcggcaagaggaacaccatctggctgtttgggcctgcaactaccgggaagaccaacatcgcggaggccatagcccacactgtgcccttctacgggtgcgtaaactggaccaatgagaactttcccttcaacgactgtgtcgacaagatggtgatctggtgggaggaggggaagatgaccgccaaggtcgtggagtcggccaaagccattctcggaggaagcaaggtgcgcgtggaccagaaatgcaagtcctcggcccagatagacccgactcccgtgatcgtcacctccaacaccaacatgtgcgccgtgattgacgggaactcaacgaccttcgaacaccagcagccgttgcaagaccggatgttcaaatttgaactcacccgccgtctggatcatgactttgggaaggtcaccaagcaggaagtcaaagactttttccggtgggcaaaggatcacgtggttgaggtggagcatgaattctacgtcaaaaagggtggagccaagaaaagacccgcccccagtgacgcagatataagtgagcccaaacgggtgcgcgagtcagttgcgcagccatcgacgtcagacgcggaagcttcgatcaactacgcagacaggtaccaaaacaaatgttctcgtcacgtgggcatgaatctgatgctgtttccctgcagacaatgcgagagaatgaatcagaattcaaatatctgcttcactcacggacagaaagactgtttagagtgctttcccgtgtcagaatctcaacccgtttctgtcgtcaaaaaggcgtatcagaaactgtgctacattcatcatatcatgggaaaggtgccagacgcttgcactgcctgcgatctggtcaatgtggatttggatgactgcatctttgaacaataa

SEQ ID NO: 6 - protein, 621 aa, adeno-associated virus 2
MPGFYEIVIKVPSDLDEHLPGISDSFVNWVAEKEWELPPDSDMDLNLIEQAPLTVAEKLQRDFLTEWRRVSKAPEALFFVQFEKGESYFHMHVLVETTGVKSMVLGRFLSQIREKLIQRIYRGIEPTLPNWFAVTKTRNGAGGGNKVVDECYIPNYLLPKTQPELQWAWTNMEQYLSACLNLTERKRLVAQHLTHVSQTQEQNKENQNPNSDAPVIRSKTSARYMELVGWLVDKGITSEKQWIQEDQASYISFNAASNSRSQIKAALDNAGKIMSLTKTAPDYLVGQQPVEDISSNRIYKILELNGYDPQYAASVFLGWATKKFGKRNTIWLFGPATTGKTNIAEAIAHTVPFYGCVNWTNENFPFNDCVDKMVIWWEEGKMTAKVVESAKAILGGSKVRVDQKCKSSAQIDPTPVIVTSNTNMCAVIDGNSTTFEHQQPLQDRMFKFELTRRLDHDFGKVTKQEVKDFFRWAKDHVVEVEHEFYVKKGGAKKRPAPSDADISEPKRVRESVAQPSTSDAEASINYADRYQNKCSRHVGMNLMLFPCRQCERMNQNSNICFTHGQKDCLECFPVSESQPVSVVKKAYQKLCYIHHIMGKVPDACTACDLVNVDLDDCIFEQ

SEQ ID NO: 7 - DNA, 1194 bp, Artificial
  AAV2 Rep52 AcMNPV optimized
  misc_feature: AcMNPV optimized Rep52 coding sequence
atggaattggtcggttggttggtggacaagggtattacctcggagaagcaatggatacaagaagatcaagcctcatacatctcgtttaatgcggcatccaactcgcgtagccaaatcaaagctgccttggacaatgcgggcaagattatgagcctgactaaaaccgcccccgactacctggtgggccagcaacccgtggaagacatttccagcaatcgcatctataagattttggagttaaacggctacgatcctcaatatgcggcttccgtatttttgggctgggcgacgaaaaagtttggcaaaagaaacaccatttggttgtttggacctgcaactacgggaaaaacaaacatagcggaggccatagcccacactgtacctttttatggctgcgttaactggaccaatgagaactttccattcaacgactgtgtcgacaagatggttatttggtgggaggaaggcaaaatgaccgctaaagtcgtggagtcggccaaagcaattttaggaggcagcaaagtgcgcgtagaccagaaatgcaaaagctctgcgcagatagacccgacaccggtgatcgttacaagcaacacgaacatgtgcgccgtgattgacggtaacagtacgacattcgaacaccaacaaccgttgcaagaccgaatgttcaaatttgaattgacgcgccgactggatcatgattttggcaaggtaacaaaacaagaagtcaaagacttctttcgttgggcaaaggatcacgttgttgaagtggaacatgaattttacgtcaaaaaaggtggtgctaagaaaagacccgccccgagtgatgcagatataagtgagcccaaacgagtgagagaatcggttgcgcagccaagcacgtcagatgcggaagcttcgataaactacgcagaccgctaccaaaacaaatgttctcgtcacgtaggcatgaacttaatgttgtttccctgcagacaatgtgagagaatgaatcagaatagtaatatctgtttcactcacggccagaaagactgtttagaatgctttccggtgtcagaatctcaacccgtttctgtcgtaaaaaaggcgtatcaaaaattatgctatattcatcatatcatgggaaaagtgccagacgcttgtactgcctgcgatctggttaatgtggatttggatgactgtatctttgaacaataa